European Patent Specification EP 3 655 529 B1, published June 25, 2025. Title: Enzyme PTE améliorée. Applicant: Chabrière, Etienne. The sequence listing filed with the application follows.

SEQUENCE LISTING (13 sequences)

SEQ ID NO: 1 - protein, 333 aa, Artificial sq.
  Sequence WT
MGDRINTVRGPITISEAGFTLTHEHICGSSAGFLRAWPEFFGSRKALAEKAVRGLRRARAAGVRTIVDVSTFDIGRDVSLLAEVSRAADVHIVAATGLWFDPPLSMRLRSVEELTQFFLREIQYGIEDTGIRAGIIKVATTGKATPFQELVLKAAARASLATGVPVTTHTAASQRDGEQQAAIFESEGLSPSRVCIGHSDDTDDLSYLTALAARGYLIGLDHIPHSAIGLEDNASASALLGIRSWQTRALLIKALIDQGYMKQILVSNDWLFGFSSYVTNIMDVMDRVNPDGMAFIPLRVIPFLREKGVPQETLAGITVTNPARFLSPTLRAS

SEQ ID NO: 2 - protein, 333 aa, Artificial sq.
  Séquence WT + 7 mutations ancestrales (T13P; I14V ; A60S ; S79R ; Y124H ; I218V ; Q258R)
MGDRINTVRGPIPVSEAGFTLTHEHICGSSAGFLRAWPEFFGSRKALAEKAVRGLRRARSAGVRTIVDVSTFDIGRDVRLLAEVSRAADVHIVAATGLWFDPPLSMRLRSVEELTQFFLREIQHGIEDTGIRAGIIKVATTGKATPFQELVLKAAARASLATGVPVTTHTAASQRDGEQQAAIFESEGLSPSRVCIGHSDDTDDLSYLTALAARGYLVGLDHIPHSAIGLEDNASASALLGIRSWQTRALLIKALIDRGYMKQILVSNDWLFGFSSYVTNIMDVMDRVNPDGMAFIPLRVIPFLREKGVPQETLAGITVTNPARFLSPTLRAS

SEQ ID NO: 3 - protein, 333 aa, Artificial sq.
  Séquence WT + 7 mutations ancestrales (T13P; I14V ; A60S ; S79R ; Y124H ; I218V ; Q258R) + 2 mutations (H225Y ; L271T)
MGDRINTVRGPIPVSEAGFTLTHEHICGSSAGFLRAWPEFFGSRKALAEKAVRGLRRARSAGVRTIVDVSTFDIGRDVRLLAEVSRAADVHIVAATGLWFDPPLSMRLRSVEELTQFFLREIQHGIEDTGIRAGIIKVATTGKATPFQELVLKAAARASLATGVPVTTHTAASQRDGEQQAAIFESEGLSPSRVCIGHSDDTDDLSYLTALAARGYLVGLDHIPYSAIGLEDNASASALLGIRSWQTRALLIKALIDRGYMKQILVSNDWTFGFSSYVTNIMDVMDRVNPDGMAFIPLRVIPFLREKGVPQETLAGITVTNPARFLSPTLRAS

SEQ ID NO: 4 - protein, 333 aa, Artificial sq.
  Séquence WT + 7 mutations ancestrales (T13P; I14V ; A60S ; S79R ; Y124H ; I218V ; Q258R) + 8 mutations (I74C ; F100V ; H222Q ; H225Y ; A238V ; L240M ; I242N ; S276L)
MGDRINTVRGPIPVSEAGFTLTHEHICGSSAGFLRAWPEFFGSRKALAEKAVRGLRRARSAGVRTIVDVSTFDCGRDVRLLAEVSRAADVHIVAATGLWVDPPLSMRLRSVEELTQFFLREIQHGIEDTGIRAGIIKVATTGKATPFQELVLKAAARASLATGVPVTTHTAASQRDGEQQAAIFESEGLSPSRVCIGHSDDTDDLSYLTALAARGYLVGLDQIPYSAIGLEDNASASVLMGNRSWQTRALLIKALIDRGYMKQILVSNDWLFGFSLYVTNIMDVMDRVNPDGMAFIPLRVIPFLREKGVPQETLAGITVTNPARFLSPTLRAS

SEQ ID NO: 5 - protein, 333 aa, Artificial sq.
  Séquence WT + 7 mutations ancestrales (T13P; I14V ; A60S ; S79R ; Y124H ; I218V ; Q258R) + 9 mutations (K45A ; A48V ; F100E ; T141N ; K153R ; H222G ; I242N ; R287S ; P310S)
MGDRINTVRGPIPVSEAGFTLTHEHICGSSAGFLRAWPEFFGSRAALVEKAVRGLRRARSAGVRTIVDVSTFDIGRDVRLLAEVSRAADVHIVAATGLWEDPPLSMRLRSVEELTQFFLREIQHGIEDTGIRAGIIKVATNGKATPFQELVLRAAARASLATGVPVTTHTAASQRDGEQQAAIFESEGLSPSRVCIGHSDDTDDLSYLTALAARGYLVGLDGIPHSAIGLEDNASASALLGNRSWQTRALLIKALIDRGYMKQILVSNDWLFGFSSYVTNIMDVMDSVNPDGMAFIPLRVIPFLREKGVSQETLAGITVTNPARFLSPTLRAS

SEQ ID NO: 6 - protein, 333 aa, Artificial sq.
  Séquence WT + 7 mutations ancestrales (T13P; I14V ; A60S ; S79R ; Y124H ; I218V ; Q258R) + 11 mutations (K45A ; A48V ; F100E ; T141N ; K153R ; G177D ; D201G ; H222G ; I242N ; Y277W ; R287S)
MGDRINTVRGPIPVSEAGFTLTHEHICGSSAGFLRAWPEFFGSRAALVEKAVRGLRRARSAGVRTIVDVSTFDIGRDVRLLAEVSRAADVHIVAATGLWEDPPLSMRLRSVEELTQFFLREIQHGIEDTGIRAGIIKVATNGKATPFQELVLRAAARASLATGVPVTTHTAASQRDDEQQAAIFESEGLSPSRVCIGHSDGTDDLSYLTALAARGYLVGLDGIPHSAIGLEDNASASALLGNRSWQTRALLIKALIDRGYMKQILVSNDWLFGFSSWVTNIMDVMDSVNPDGMAFIPLRVIPFLREKGVPQETLAGITVTNPARFLSPTLRAS

SEQ ID NO: 7 - protein, 333 aa, Artificial sq.
  Séquence WT + 7 mutations ancestrales (T13P; I14V ; A60S ; S79R ; Y124H ; I218V ; Q258R) + 12 mutations (K45A ; A48V ; I74A ; F100E ; T141N ; K153R ; G177D ; D201G ; H222G ; I242N ; Y277W ; R287S)
MGDRINTVRGPIPVSEAGFTLTHEHICGSSAGFLRAWPEFFGSRAALVEKAVRGLRRARSAGVRTIVDVSTFDAGRDVRLLAEVSRAADVHIVAATGLWEDPPLSMRLRSVEELTQFFLREIQHGIEDTGIRAGIIKVATNGKATPFQELVLRAAARASLATGVPVTTHTAASQRDDEQQAAIFESEGLSPSRVCIGHSDGTDDLSYLTALAARGYLVGLDGIPHSAIGLEDNASASALLGNRSWQTRALLIKALIDRGYMKQILVSNDWLFGFSSWVTNIMDVMDSVNPDGMAFIPLRVIPFLREKGVPQETLAGITVTNPARFLSPTLRAS

SEQ ID NO: 8 - protein, 333 aa, Artificial sq.
  Séquence WT + 7 mutations ancestrales (T13P; I14V ; A60S ; S79R ; Y124H ; I218V ; Q258R) + 13 mutations (K45A ; A48M ; F100E ; T141N ; K153R ; G177D ; D201G ; H222G; A238S ; L239W ; I242N ; Y277W ; R287S)
MGDRINTVRGPIPVSEAGFTLTHEHICGSSAGFLRAWPEFFGSRAALMEKAVRGLRRARSAGVRTIVDVSTFDIGRDVRLLAEVSRAADVHIVAATGLWEDPPLSMRLRSVEELTQFFLREIQHGIEDTGIRAGIIKVATNGKATPFQELVLRAAARASLATGVPVTTHTAASQRDDEQQAAIFESEGLSPSRVCIGHSDGTDDLSYLTALAARGYLVGLDGIPHSAIGLEDNASASSWLGNRSWQTRALLIKALIDRGYMKQILVSNDWLFGFSSWVTNIMDVMDSVNPDGMAFIPLRVIPFLREKGVPQETLAGITVTNPARFLSPTLRAS

SEQ ID NO: 9 - protein, 333 aa, Artificial sq.
  Séquence WT + 7 mutations ancestrales (T13P; I14V ; A60S ; S79R ; Y124H ; I218V ; Q258R) + 174 mutations (K45A ; A48M ; I74A ; F100E ; T141N ; K153R ; G177D ; D201G ; H222G ; A238S ; L239W ; I242N ; Y277W ; R287S)
MGDRINTVRGPIPVSEAGFTLTHEHICGSSAGFLRAWPEFFGSRAALMEKAVRGLRRARSAGVRTIVDVSTFDAGRDVRLLAEVSRAADVHIVAATGLWEDPPLSMRLRSVEELTQFFLREIQHGIEDTGIRAGIIKVATNGKATPFQELVLRAAARASLATGVPVTTHTAASQRDDEQQAAIFESEGLSPSRVCIGHSDGTDDLSYLTALAARGYLVGLDGIPHSAIGLEDNASASSWLGNRSWQTRALLIKALIDRGYMKQILVSNDWLFGFSSWVTNIMDVMDSVNPDGMAFIPLRVIPFLREKGVPQETLAGITVTNPARFLSPTLRAS

SEQ ID NO: 10 - protein, 333 aa, Artificial sq.
  Séquence WT + 7 mutations ancestrales (T13P; I14V ; A60S ; S79R ; Y124H ; I218V ; Q258R) + 14 mutations (K45A ; A48M ; F100E ; T141N ; K153R ; G177D ; D201G ; H222G ; S235M ; A238S ; L239W ; I242N ; Y277W ; R287S)
MGDRINTVRGPIPVSEAGFTLTHEHICGSSAGFLRAWPEFFGSRAALMEKAVRGLRRARSAGVRTIVDVSTFDIGRDVRLLAEVSRAADVHIVAATGLWEDPPLSMRLRSVEELTQFFLREIQHGIEDTGIRAGIIKVATNGKATPFQELVLRAAARASLATGVPVTTHTAASQRDDEQQAAIFESEGLSPSRVCIGHSDGTDDLSYLTALAARGYLVGLDGIPHSAIGLEDNAMASSWLGNRSWQTRALLIKALIDRGYMKQILVSNDWLFGFSSWVTNIMDVMDSVNPDGMAFIPLRVIPFLREKGVPQETLAGITVTNPARFLSPTLRAS

SEQ ID NO: 11 - protein, 333 aa, Artificial sq.
  Séquence WT + 7 mutations ancestrales (T13P; I14V ; A60S ; S79R ; Y124H ; I218V ; Q258R) + 15 mutations (K45A ; A48M ; I74A ; F100E ; T141N ; K153R ; G177D ; D201G ; H222G ; S235M ; A238S ; L239W ; I242N ; Y277W ; R287S)
MGDRINTVRGPIPVSEAGFTLTHEHICGSSAGFLRAWPEFFGSRAALMEKAVRGLRRARSAGVRTIVDVSTFDAGRDVRLLAEVSRAADVHIVAATGLWEDPPLSMRLRSVEELTQFFLREIQHGIEDTGIRAGIIKVATNGKATPFQELVLRAAARASLATGVPVTTHTAASQRDDEQQAAIFESEGLSPSRVCIGHSDGTDDLSYLTALAARGYLVGLDGIPHSAIGLEDNAMASSWLGNRSWQTRALLIKALIDRGYMKQILVSNDWLFGFSSWVTNIMDVMDSVNPDGMAFIPLRVIPFLREKGVPQETLAGITVTNPARFLSPTLRAS

SEQ ID NO: 12 - protein, 333 aa, Artificial sq.
  Séquence WT + 7 mutations ancestrales (T13P; I14V ; A60S ; S79R ; Y124H ; I218V ; Q258R) + 15 mutations (K45A ; A48M ; I74C ; F100E ; T141N ; K153R ; G177D ; D201G ; H222G ; S235M ; A238S ; L239W ; I242N ; Y277W ; R287S)
MGDRINTVRGPIPVSEAGFTLTHEHICGSSAGFLRAWPEFFGSRAALMEKAVRGLRRARSAGVRTIVDVSTFDCGRDVRLLAEVSRAADVHIVAATGLWEDPPLSMRLRSVEELTQFFLREIQHGIEDTGIRAGIIKVATNGKATPFQELVLRAAARASLATGVPVTTHTAASQRDDEQQAAIFESEGLSPSRVCIGHSDGTDDLSYLTALAARGYLVGLDGIPHSAIGLEDNAMASSWLGNRSWQTRALLIKALIDRGYMKQILVSNDWLFGFSSWVTNIMDVMDSVNPDGMAFIPLRVIPFLREKGVPQETLAGITVTNPARFLSPTLRAS

SEQ ID NO: 13 - protein, 333 aa, Artificial sq.
  Séquence WT + 8 mutations (I74C ; F100V ; H222Q ; H225Y ; A238V ; L240M ; I242N ; S276L)
MGDRINTVRGPITISEAGFTLTHEHICGSSAGFLRAWPEFFGSRKALAEKAVRGLRRARAAGVRTIVDVSTFDCGRDVSLLAEVSRAADVHIVAATGLWVDPPLSMRLRSVEELTQFFLREIQYGIEDTGIRAGIIKVATTGKATPFQELVLKAAARASLATGVPVTTHTAASQRDGEQQAAIFESEGLSPSRVCIGHSDDTDDLSYLTALAARGYLIGLDQIPYSAIGLEDNASASVLMGNRSWQTRALLIKALIDQGYMKQILVSNDWLFGFSLYVTNIMDVMDRVNPDGMAFIPLRVIPFLREKGVPQETLAGITVTNPARFLSPTLRAS